European Patent Application EP 4 509 128 A1, published February 19, 2025. Title: 줄기세포로부터 분리된 세포외 소포체 및 이의 용도. Applicant: 인엑소플랫. The sequence listing filed with the application follows.

SEQUENCE LISTING (14 sequences)

SEQ ID NO: 1 - DNA, 23 bp, synthetic construct
  misc_feature 1..23: note = GAPDH_Forward Primer
  source 1..23: mol_type = other DNA
catcactgccacccagaagactg

SEQ ID NO: 2 - DNA, 23 bp, synthetic construct
  misc_feature 1..23: note = GAPDH_Reverse Primer
  source 1..23: mol_type = other DNA
atgccagtgagcttcccgttcag

SEQ ID NO: 3 - DNA, 21 bp, synthetic construct
  misc_feature 1..21: note = IL-6_Forward Primer
  source 1..21: mol_type = other DNA
agttgccttcttgggactgat

SEQ ID NO: 4 - DNA, 21 bp, synthetic construct
  misc_feature 1..21: note = IL-6_Reverse Primer
  source 1..21: mol_type = other DNA
tccacgatttcccagagaaca

SEQ ID NO: 5 - DNA, 20 bp, synthetic construct
  misc_feature 1..20: note = IL-12_Forward Primer
  source 1..20: mol_type = other DNA
aggtcacactggaccaaagg

SEQ ID NO: 6 - DNA, 20 bp, synthetic construct
  misc_feature 1..20: note = IL-12_Reverse Primer
  source 1..20: mol_type = other DNA
tggtttgatgatgtccctga

SEQ ID NO: 7 - DNA, 22 bp, synthetic construct
  misc_feature 1..22: note = IL-1beta_Forward Primer
  source 1..22: mol_type = other DNA
ttcctgttgtctacaccaatgc

SEQ ID NO: 8 - DNA, 22 bp, synthetic construct
  misc_feature 1..22: note = IL-1beta_Reverse Primer
  source 1..22: mol_type = other DNA
cgggctttaagtgagtaggaga

SEQ ID NO: 9 - DNA, 20 bp, synthetic construct
  misc_feature 1..20: note = TNF-alpha_Forward Primer
  source 1..20: mol_type = other DNA
acggcatggatctcaaagac

SEQ ID NO: 10 - DNA, 20 bp, synthetic construct
  misc_feature 1..20: note = TNF-alpha_Reverse Primer
  source 1..20: mol_type = other DNA
gtgggtgaggagcacgtagt

SEQ ID NO: 11 - DNA, 24 bp, synthetic construct
  misc_feature 1..24: note = NOS2_Forward Primer
  source 1..24: mol_type = other DNA
gaactgtagcacagcacaggaaat

SEQ ID NO: 12 - DNA, 21 bp, synthetic construct
  misc_feature 1..21: note = NOS2_Reverse Primer
  source 1..21: mol_type = other DNA
cgtaccggatgagctgtgaat

SEQ ID NO: 13 - DNA, 27 bp, synthetic construct
  misc_feature 1..27: note = COX2_Forward Primer
  source 1..27: mol_type = other DNA
cagtttatgttgtctgtccagagtttc

SEQ ID NO: 14 - DNA, 21 bp, synthetic construct
  misc_feature 1..21: note = COX2_Reverse Primer
  source 1..21: mol_type = other DNA
ccagcacttcacccatcagtt